European Patent Application EP 4 119 127 A1, published January 18, 2023. Title: IMMUNE AGONIST COMPLEX, AND PREPARATION AND APPLICATION THEREOF. Applicant: Hangzhou Xingao Biotechnology Co., Ltd. The sequence listing filed with the application follows.

SEQUENCE LISTING (4 sequences)

SEQ ID NO: 1 - protein, 23 aa, Artificial Sequence
  synthesis
HGLASTLTRWAHYNALIRAFGGG

SEQ ID NO: 2 - protein, 8 aa, Artificial Sequence
  synthesis
CHAIYPRH

SEQ ID NO: 3 - DNA, 17 bp, Artificial Sequence
  synthesis
agaagcggaatgggagc

SEQ ID NO: 4 - DNA, 17 bp, Artificial Sequence
  synthesis
gaggtgggtgggaagga